European Patent Application EP 4 212 210 A1, published July 19, 2023. Title: ANTI-SORTILIN ANTIBODIES AND METHODS OF USE THEREOF. Applicant: Alector LLC. The sequence listing filed with the application follows.

SEQUENCE LISTING (146 sequences)

SEQ ID NO: 1 - protein, 10 aa, synthetic construct
  REGION 1..10: note = Synthetic Construct
YSISSGYYWG

SEQ ID NO: 2 - protein, 16 aa, synthetic construct
  REGION 1..16: note = Synthetic Construct
TIYHSGSTYYNPSLKS

SEQ ID NO: 3 - protein, 16 aa, synthetic construct
  REGION 1..16: note = Synthetic Construct
TIYHSGSTYYNPSLES

SEQ ID NO: 4 - protein, 16 aa, synthetic construct
  REGION 1..16: note = Synthetic Construct
  VARIANT 15: note = Xaa = Lys or Glu
TIYHSGSTYYNPSLXS

SEQ ID NO: 5 - protein, 15 aa, synthetic construct
  REGION 1..15: note = Synthetic Construct
ARQGSIQQGYYGMDV

SEQ ID NO: 6 - protein, 15 aa, synthetic construct
  REGION 1..15: note = Synthetic Construct
ARQGSIKQGYYGMDV

SEQ ID NO: 7 - protein, 15 aa, synthetic construct
  REGION 1..15: note = Synthetic Construct
  VARIANT 7: note = Xaa = Gln or Lys
ARQGSIXQGYYGMDV

SEQ ID NO: 8 - protein, 16 aa, synthetic construct
  REGION 1..16: note = Synthetic Construct
RSSQSLLRSNGYNYLD

SEQ ID NO: 9 - protein, 16 aa, synthetic construct
  REGION 1..16: note = Synthetic Construct
RSSQSLLRSTGYNYLD

SEQ ID NO: 10 - protein, 16 aa, synthetic construct
  REGION 1..16: note = Synthetic Construct
RSSQSLLRSSGYNYLD

SEQ ID NO: 11 - protein, 16 aa, synthetic construct
  REGION 1..16: note = Synthetic Construct
RSSQSLLRSGGYNYLD

SEQ ID NO: 12 - protein, 16 aa, synthetic construct
  REGION 1..16: note = Synthetic Construct
RSSQSLLRSRGYNYLD

SEQ ID NO: 13 - protein, 16 aa, synthetic construct
  REGION 1..16: note = Synthetic Construct
RSSQSLLRSDGYNYLD

SEQ ID NO: 14 - protein, 16 aa, synthetic construct
  REGION 1..16: note = Synthetic Construct
RSSQSLLRSHGYNYLD

SEQ ID NO: 15 - protein, 16 aa, synthetic construct
  REGION 1..16: note = Synthetic Construct
RSSQSLLRSKGYNYLD

SEQ ID NO: 16 - protein, 16 aa, synthetic construct
  REGION 1..16: note = Synthetic Construct
RSSQSLLRSQGYNYLD

SEQ ID NO: 17 - protein, 16 aa, synthetic construct
  REGION 1..16: note = Synthetic Construct
RSSQSLLRSYGYNYLD

SEQ ID NO: 18 - protein, 16 aa, synthetic construct
  REGION 1..16: note = Synthetic Construct
RSSQSLLRSEGYNYLD

SEQ ID NO: 19 - protein, 16 aa, synthetic construct
  REGION 1..16: note = Synthetic Construct
RSSQSLLRSWGYNYLD

SEQ ID NO: 20 - protein, 16 aa, synthetic construct
  REGION 1..16: note = Synthetic Construct
RSSQSLLRSFGYNYLD

SEQ ID NO: 21 - protein, 16 aa, synthetic construct
  REGION 1..16: note = Synthetic Construct
RSSQSLLRSIGYNYLD

SEQ ID NO: 22 - protein, 16 aa, synthetic construct
  REGION 1..16: note = Synthetic Construct
RSSQSLLRSVGYNYLD

SEQ ID NO: 23 - protein, 16 aa, synthetic construct
  REGION 1..16: note = Synthetic Construct
RSSQSLLRSAGYNYLD

SEQ ID NO: 24 - protein, 16 aa, synthetic construct
  REGION 1..16: note = Synthetic Construct
RSSQSLLRSMGYNYLD

SEQ ID NO: 25 - protein, 16 aa, synthetic construct
  REGION 1..16: note = Synthetic Construct
RSSQSLLRSLGYNYLD

SEQ ID NO: 26 - protein, 16 aa, synthetic construct
  REGION 1..16: note = Synthetic Construct
RSSQSLLHSNGYNYLD

SEQ ID NO: 27 - protein, 16 aa, synthetic construct
  REGION 1..16: note = Synthetic Construct
RSSQGLLRSNGYNYLD

SEQ ID NO: 28 - protein, 16 aa, synthetic construct
  REGION 1..16: note = Synthetic Construct
  VARIANT 5: note = Xaa = Ser or Gly
  VARIANT 8: note = Xaa = Arg or His
  VARIANT 10: note = Xaa = Asn, Thr, Ser, Gly, Arg, Asp, His, Lys, Gln, Tyr, Glu, Trp, Phe, Ile, Val, Ala, Met, or Leu
RSSQXLLXSXGYNYLD

SEQ ID NO: 29 - protein, 7 aa, synthetic construct
  REGION 1..7: note = Synthetic Construct
LGSNRAS

SEQ ID NO: 30 - protein, 7 aa, synthetic construct
  REGION 1..7: note = Synthetic Construct
LGSNRVS

SEQ ID NO: 31 - protein, 7 aa, synthetic construct
  REGION 1..7: note = Synthetic Construct
  VARIANT 6: note = Xaa = Ala or Val
LGSNRXS

SEQ ID NO: 32 - protein, 9 aa, synthetic construct
  REGION 1..9: note = Synthetic Construct
MQQQEAPLT

SEQ ID NO: 33 - protein, 9 aa, synthetic construct
  REGION 1..9: note = Synthetic Construct
MQQQETPLT

SEQ ID NO: 34 - protein, 9 aa, synthetic construct
  REGION 1..9: note = Synthetic Construct
  VARIANT 6: note = Xaa = Ala or Thr
MQQQEXPLT

SEQ ID NO: 35 - protein, 26 aa, synthetic construct
  REGION 1..26: note = Synthetic Construct
QVQLQESGPGLVKPSETLSLTCAVSG

SEQ ID NO: 36 - protein, 14 aa, synthetic construct
  REGION 1..14: note = Synthetic Construct
WIRQPPGKGLEWIG

SEQ ID NO: 37 - protein, 30 aa, synthetic construct
  REGION 1..30: note = Synthetic Construct
QVTISVDTSKNQFSLELSSVTAADTAVYYC

SEQ ID NO: 38 - protein, 30 aa, synthetic construct
  REGION 1..30: note = Synthetic Construct
RVTISVDTSKNQFSLKLSSVTAADTAVYYC

SEQ ID NO: 39 - protein, 30 aa, synthetic construct
  REGION 1..30: note = Synthetic Construct
  VARIANT 1: note = Xaa = Gln or Arg
  VARIANT 16: note = Xaa = Glu or Lys
XVTISVDTSKNQFSLXLSSVTAADTAVYYC

SEQ ID NO: 40 - protein, 11 aa, synthetic construct
  REGION 1..11: note = Synthetic Construct
WGQGTTVTVSS

SEQ ID NO: 41 - protein, 23 aa, synthetic construct
  REGION 1..23: note = Synthetic Construct
DIVMTQSPLSLPVTPGEPASISC

SEQ ID NO: 42 - protein, 23 aa, synthetic construct
  REGION 1..23: note = Synthetic Construct
DIVMTQSPLSLPVTPGGPASISC

SEQ ID NO: 43 - protein, 23 aa, synthetic construct
  REGION 1..23: note = Synthetic Construct
DIVMTQSPLSLPVTPGESASISC

SEQ ID NO: 44 - protein, 23 aa, synthetic construct
  REGION 1..23: note = Synthetic Construct
  VARIANT 17: note = Xaa = Glu or Gly
  VARIANT 18: note = Xaa = Pro or Ser
DIVMTQSPLSLPVTPGXXASISC

SEQ ID NO: 45 - protein, 15 aa, synthetic construct
  REGION 1..15: note = Synthetic Construct
WYLQKPGQSPQLLIY

SEQ ID NO: 46 - protein, 15 aa, synthetic construct
  REGION 1..15: note = Synthetic Construct
WYLQKPGQPPQLLIY

SEQ ID NO: 47 - protein, 15 aa, synthetic construct
  REGION 1..15: note = Synthetic Construct
  VARIANT 9: note = Xaa = Ser or Pro
WYLQKPGQXPQLLIY

SEQ ID NO: 48 - protein, 32 aa, synthetic construct
  REGION 1..32: note = Synthetic Construct
GVPDRFSGSGSGTDFTLKISRAEAEDVGVYYC

SEQ ID NO: 49 - protein, 32 aa, synthetic construct
  REGION 1..32: note = Synthetic Construct
GVPDRFSGSGSGTDFTLKISRVEAEDVGVYYC

SEQ ID NO: 50 - protein, 32 aa, synthetic construct
  REGION 1..32: note = Synthetic Construct
GVPDRFSGSGSGTDFTLKISRVEAEDVGAYYC

SEQ ID NO: 51 - protein, 32 aa, synthetic construct
  REGION 1..32: note = Synthetic Construct
GVPDRLSGSGSGTDFTLKISRVEAEDVGVYYC

SEQ ID NO: 52 - protein, 32 aa, synthetic construct
  REGION 1..32: note = Synthetic Construct
  VARIANT 6: note = Xaa = Phe or Leu
  VARIANT 22: note = Xaa = Ala or Val
  VARIANT 29: note = Xaa = Val or Ala
GVPDRXSGSGSGTDFTLKISRXEAEDVGXYYC

SEQ ID NO: 53 - protein, 10 aa, synthetic construct
  REGION 1..10: note = Synthetic Construct
FGGGTKVEIK

SEQ ID NO: 54 - protein, 122 aa, synthetic construct
  REGION 1..122: note = Synthetic Construct
QVQLQESGPGLVKPSETLSLTCAVSGYSISSGYYWGWIRQPPGKGLEWIGTIYHSGSTYYNPSLKSQVTISVDTSKNQFSLELSSVTAADTAVYYCARQGSIQQGYYGMDVWGQGTTVTVSS

SEQ ID NO: 55 - protein, 122 aa, synthetic construct
  REGION 1..122: note = Synthetic Construct
QVQLQESGPGLVKPSETLSLTCAVSGYSISSGYYWGWIRQPPGKGLEWIGTIYHSGSTYYNPSLESRVTISVDTSKNQFSLKLSSVTAADTAVYYCARQGSIQQGYYGMDVWGQGTTVTVSS

SEQ ID NO: 56 - protein, 122 aa, synthetic construct
  REGION 1..122: note = Synthetic Construct
QVQLQESGPGLVKPSETLSLTCAVSGYSISSGYYWGWIRQPPGKGLEWIGTIYHSGSTYYNPSLKSRVTISVDTSKNQFSLKLSSVTAADTAVYYCARQGSIKQGYYGMDVWGQGTTVTVSS

SEQ ID NO: 57 - protein, 112 aa, synthetic construct
  REGION 1..112: note = Synthetic Construct
DIVMTQSPLSLPVTPGEPASISCRSSQSLLRSNGYNYLDWYLQKPGQSPQLLIYLGSNRASGVPDRFSGSGSGTDFTLKISRAEAEDVGVYYCMQQQEAPLTFGGGTKVEIK

SEQ ID NO: 58 - protein, 112 aa, synthetic construct
  REGION 1..112: note = Synthetic Construct
DIVMTQSPLSLPVTPGEPASISCRSSQSLLRSNGYNYLDWYLQKPGQSPQLLIYLGSNRASGVPDRFSGSGSGTDFTLKISRVEAEDVGVYYCMQQQEAPLTFGGGTKVEIK

SEQ ID NO: 59 - protein, 112 aa, synthetic construct
  REGION 1..112: note = Synthetic Construct
DIVMTQSPLSLPVTPGEPASISCRSSQSLLRSNGYNYLDWYLQKPGQPPQLLIYLGSNRVSGVPDRFSGSGSGTDFTLKISRVEAEDVGVYYCMQQQETPLTFGGGTKVEIK

SEQ ID NO: 60 - protein, 112 aa, synthetic construct
  REGION 1..112: note = Synthetic Construct
DIVMTQSPLSLPVTPGEPASISCRSSQSLLRSTGYNYLDWYLQKPGQSPQLLIYLGSNRASGVPDRFSGSGSGTDFTLKISRAEAEDVGVYYCMQQQEAPLTFGGGTKVEIK

SEQ ID NO: 61 - protein, 112 aa, synthetic construct
  REGION 1..112: note = Synthetic Construct
DIVMTQSPLSLPVTPGEPASISCRSSQSLLRSSGYNYLDWYLQKPGQSPQLLIYLGSNRASGVPDRFSGSGSGTDFTLKISRAEAEDVGVYYCMQQQEAPLTFGGGTKVEIK

SEQ ID NO: 62 - protein, 112 aa, synthetic construct
  REGION 1..112: note = Synthetic Construct
DIVMTQSPLSLPVTPGEPASISCRSSQSLLRSGGYNYLDWYLQKPGQSPQLLIYLGSNRASGVPDRFSGSGSGTDFTLKISRAEAEDVGVYYCMQQQEAPLTFGGGTKVEIK

SEQ ID NO: 63 - protein, 112 aa, synthetic construct
  REGION 1..112: note = Synthetic Construct
DIVMTQSPLSLPVTPGEPASISCRSSQSLLRSRGYNYLDWYLQKPGQSPQLLIYLGSNRASGVPDRFSGSGSGTDFTLKISRAEAEDVGVYYCMQQQEAPLTFGGGTKVEIK

SEQ ID NO: 64 - protein, 112 aa, synthetic construct
  REGION 1..112: note = Synthetic Construct
DIVMTQSPLSLPVTPGEPASISCRSSQSLLRSDGYNYLDWYLQKPGQSPQLLIYLGSNRASGVPDRFSGSGSGTDFTLKISRAEAEDVGVYYCMQQQEAPLTFGGGTKVEIK

SEQ ID NO: 65 - protein, 112 aa, synthetic construct
  REGION 1..112: note = Synthetic Construct
DIVMTQSPLSLPVTPGEPASISCRSSQSLLRSHGYNYLDWYLQKPGQSPQLLIYLGSNRASGVPDRFSGSGSGTDFTLKISRAEAEDVGVYYCMQQQEAPLTFGGGTKVEIK

SEQ ID NO: 66 - protein, 112 aa, synthetic construct
  REGION 1..112: note = Synthetic Construct
DIVMTQSPLSLPVTPGEPASISCRSSQSLLRSKGYNYLDWYLQKPGQSPQLLIYLGSNRASGVPDRFSGSGSGTDFTLKISRAEAEDVGVYYCMQQQEAPLTFGGGTKVEIK

SEQ ID NO: 67 - protein, 112 aa, synthetic construct
  REGION 1..112: note = Synthetic Construct
DIVMTQSPLSLPVTPGEPASISCRSSQSLLRSQGYNYLDWYLQKPGQSPQLLIYLGSNRASGVPDRFSGSGSGTDFTLKISRAEAEDVGVYYCMQQQEAPLTFGGGTKVEIK

SEQ ID NO: 68 - protein, 112 aa, synthetic construct
  REGION 1..112: note = Synthetic Construct
DIVMTQSPLSLPVTPGEPASISCRSSQSLLRSYGYNYLDWYLQKPGQSPQLLIYLGSNRASGVPDRFSGSGSGTDFTLKISRAEAEDVGVYYCMQQQEAPLTFGGGTKVEIK

SEQ ID NO: 69 - protein, 112 aa, synthetic construct
  REGION 1..112: note = Synthetic Construct
DIVMTQSPLSLPVTPGEPASISCRSSQSLLRSEGYNYLDWYLQKPGQSPQLLIYLGSNRASGVPDRFSGSGSGTDFTLKISRAEAEDVGVYYCMQQQEAPLTFGGGTKVEIK

SEQ ID NO: 70 - protein, 112 aa, synthetic construct
  REGION 1..112: note = Synthetic Construct
DIVMTQSPLSLPVTPGEPASISCRSSQSLLRSWGYNYLDWYLQKPGQSPQLLIYLGSNRASGVPDRFSGSGSGTDFTLKISRAEAEDVGVYYCMQQQEAPLTFGGGTKVEIK

SEQ ID NO: 71 - protein, 112 aa, synthetic construct
  REGION 1..112: note = Synthetic Construct
DIVMTQSPLSLPVTPGEPASISCRSSQSLLRSFGYNYLDWYLQKPGQSPQLLIYLGSNRASGVPDRFSGSGSGTDFTLKISRAEAEDVGVYYCMQQQEAPLTFGGGTKVEIK

SEQ ID NO: 72 - protein, 112 aa, synthetic construct
  REGION 1..112: note = Synthetic Construct
DIVMTQSPLSLPVTPGEPASISCRSSQSLLRSIGYNYLDWYLQKPGQSPQLLIYLGSNRASGVPDRFSGSGSGTDFTLKISRAEAEDVGVYYCMQQQEAPLTFGGGTKVEIK

SEQ ID NO: 73 - protein, 112 aa, synthetic construct
  REGION 1..112: note = Synthetic Construct
DIVMTQSPLSLPVTPGEPASISCRSSQSLLRSVGYNYLDWYLQKPGQSPQLLIYLGSNRASGVPDRFSGSGSGTDFTLKISRAEAEDVGVYYCMQQQEAPLTFGGGTKVEIK

SEQ ID NO: 74 - protein, 112 aa, synthetic construct
  REGION 1..112: note = Synthetic Construct
DIVMTQSPLSLPVTPGEPASISCRSSQSLLRSAGYNYLDWYLQKPGQSPQLLIYLGSNRASGVPDRFSGSGSGTDFTLKISRAEAEDVGVYYCMQQQEAPLTFGGGTKVEIK

SEQ ID NO: 75 - protein, 112 aa, synthetic construct
  REGION 1..112: note = Synthetic Construct
DIVMTQSPLSLPVTPGEPASISCRSSQSLLRSMGYNYLDWYLQKPGQSPQLLIYLGSNRASGVPDRFSGSGSGTDFTLKISRAEAEDVGVYYCMQQQEAPLTFGGGTKVEIK

SEQ ID NO: 76 - protein, 112 aa, synthetic construct
  REGION 1..112: note = Synthetic Construct
DIVMTQSPLSLPVTPGEPASISCRSSQSLLRSLGYNYLDWYLQKPGQSPQLLIYLGSNRASGVPDRFSGSGSGTDFTLKISRAEAEDVGVYYCMQQQEAPLTFGGGTKVEIK

SEQ ID NO: 77 - protein, 112 aa, synthetic construct
  REGION 1..112: note = Synthetic Construct
DIVMTQSPLSLPVTPGEPASISCRSSQSLLRSNGYNYLDWYLQKPGQSPQLLIYLGSNRASGVPDRFSGSGSGTDFTLKISRVEAEDVGAYYCMQQQEAPLTFGGGTKVEIK

SEQ ID NO: 78 - protein, 112 aa, synthetic construct
  REGION 1..112: note = Synthetic Construct
DIVMTQSPLSLPVTPGGPASISCRSSQSLLRSNGYNYLDWYLQKPGQSPQLLIYLGSNRASGVPDRLSGSGSGTDFTLKISRVEAEDVGVYYCMQQQETPLTFGGGTKVEIK

SEQ ID NO: 79 - protein, 112 aa, synthetic construct
  REGION 1..112: note = Synthetic Construct
DIVMTQSPLSLPVTPGEPASISCRSSQSLLHSNGYNYLDWYLQKPGQSPQLLIYLGSNRASGVPDRFSGSGSGTDFTLKISRVEAEDVGVYYCMQQQETPLTFGGGTKVEIK

SEQ ID NO: 80 - protein, 112 aa, synthetic construct
  REGION 1..112: note = Synthetic Construct
DIVMTQSPLSLPVTPGESASISCRSSQGLLRSNGYNYLDWYLQKPGQSPQLLIYLGSNRASGVPDRFSGSGSGTDFTLKISRVEAEDVGVYYCMQQQEAPLTFGGGTKVEIK

SEQ ID NO: 81 - protein, 831 aa, Homo sapiens
MERPWGAADGLSRWPHGLGLLLLLQLLPPSTLSQDRLDAPPPPAAPLPRWSGPIGVSWGLRAAAAGGAFPRGGRWRRSAPGEDEECGRVRDFVAKLANNTHQHVFDDLRGSVSLSWVGDSTGVILVLTTFHVPLVIMTFGQSKLYRSEDYGKNFKDITDLINNTFIRTEFGMAIGPENSGKVVLTAEVSGGSRGGRIFRSSDFAKNFVQTDLPFHPLTQMMYSPQNSDYLLALSTENGLWVSKNFGGKWEEIHKAVCLAKWGSDNTIFFTTYANGSCKADLGALELWRTSDLGKSFKTIGVKIYSFGLGGRFLFASVMADKDTTRRIHVSTDQGDTWSMAQLPSVGQEQFYSILAANDDMVFMHVDEPGDTGFGTIFTSDDRGIVYSKSLDRHLYTTTGGETDFTNVTSLRGVYITSVLSEDNSIQTMITFDQGGRWTHLRKPENSECDATAKNKNECSLHIHASYSISQKLNVPMAPLSEPNAVGIVIAHGSVGDAISVMVPDVYISDDGGYSWTKMLEGPHYYTILDSGGIIVAIEHSSRPINVIKFSTDEGQCWQTYTFTRDPIYFTGLASEPGARSMNISIWGFTESFLTSQWVSYTIDFKDILERNCEEKDYTIWLAHSTDPEDYEDGCILGYKEQFLRLRKSSVCQNGRDYVVTKQPSICLCSLEDFLCDFGYYRPENDSKCVEQPELKGHDLEFCLYGREEHLTTNGYRKIPGDKCQGGVNPVREVKDLKKKCTSNFLSPEKQNSKSNSVPIILAIVGLMLVTVVAGVLIVKKYVCGGRFLVHRYSVLQQHAEANGVDGVDALDTASHTNKSGYHDDSDEDLLE

SEQ ID NO: 82 - protein, 825 aa, Mus musculus
MERPRGAADGLLRWPLGLLLLLQLLPPAAVGQDRLDAPPPPAPPLLRWAGPVGVSWGLRAAAPGGPVPRAGRWRRGAPAEDQDCGRLPDFIAKLTNNTHQHVFDDLSGSVSLSWVGDSTGVILVLTTFQVPLVIVSFGQSKLYRSEDYGKNFKDITNLINNTFIRTEFGMAIGPENSGKVILTAEVSGGSRGGRVFRSSDFAKNFVQTDLPFHPLTQMMYSPQNSDYLLALSTENGLWVSKNFGEKWEEIHKAVCLAKWGPNNIIFFTTHVNGSCKADLGALELWRTSDLGKTFKTIGVKIYSFGLGGRFLFASVMADKDTTRRIHVSTDQGDTWSMAQLPSVGQEQFYSILAANEDMVFMHVDEPGDTGFGTIFTSDDRGIVYSKSLDRHLYTTTGGETDFTNVTSLRGVYITSTLSEDNSIQSMITFDQGGRWEHLRKPENSKCDATAKNKNECSLHIHASYSISQKLNVPMAPLSEPNAVGIVIAHGSVGDAISVMVPDVYISDDGGYSWAKMLEGPHYYTILDSGGIIVAIEHSNRPINVIKFSTDEGQCWQSYVFTQEPIYFTGLASEPGARSMNISIWGFTESFITRQWVSYTVDFKDILERNCEEDDYTTWLAHSTDPGDYKDGCILGYKEQFLRLRKSSVCQNGRDYVVAKQPSVCPCSLEDFLCDFGYFRPENASECVEQPELKGHELEFCLYGKEEHLTTNGYRKIPGDKCQGGMNPAREVKDLKKKCTSNFLNPTKQNSKSNSVPIILAIVGLMLVTVVAGVLIVKKYVCGGRFLVHRYSVLQQHAEADGVEALDSTSHAKSGYHDDSDEDLLE

SEQ ID NO: 83 - protein, 825 aa, Rattus norvegicus
MERPRGAADGLLRWPLGLLLLLQLLPPAAVGQDRLDAPPPPAPPLLRWAGPVGVSWGLRAAAPGGPVPRAGRWRRGAPAEDQDCGRLPDFIAKLTNNTHQHVFDDLSGSVSLSWVGDSTGVILVLTTFQVPLVIVSFGQSKLYRSEDYGKNFKDITNLINNTFIRTEFGMAIGPENSGKVILTAEVSGGSRGGRVFRSSDFAKNFVQTDLPFHPLTQMMYSPQNSDYLLALSTENGLWVSKNFGEKWEEIHKAVCLAKWGPNNIIFFTTHVNGSCKADLGALELWRTSDLGKTFKTIGVKIYSFGLGGRFLFASVMADKDTTRRIHVSTDQGDTWSMAQLPSVGQEQFYSILAANDDMVFMHVDEPGDTGFGTIFTSDDRGIVYSKSLDRHLYTTTGGETDFTNVTSLRGVYITSTLSEDNSIQSMITFDQGGRWEHLQKPENSKCDATAKNKNECSLHIHASYSISQKLNVPMAPLSEPNAVGIVIAHGSVGDAISVMVPDVYISDDGGYSWAKMLEGPHYYTILDSGGIIVAIEHSNRPINVIKFSTDEGQCWQSYVFSQEPVYFTGLASEPGARSMNISIWGFTESFLTRQWVSYTIDFKDILERNCEENDYTTWLAHSTDPGDYKDGCILGYKEQFLRLRKSSVCQNGRDYVVAKQPSICPCSLEDFLCDFGYFRPENASECVEQPELKGHELEFCLYGKEEHLTTNGYRKIPGDRCQGGMNPAREVKDLKKKCTSNFLNPKKQNSKSSSVPIILAIVGLMLVTVVAGVLIVKKYVCGGRFLVHRYSVLQQHAEADGVEALDTASHAKSGYHDDSDEDLLE

SEQ ID NO: 84-85 - skipped (2 entries)

SEQ ID NO: 86 - protein, 8 aa, synthetic construct
  REGION 1..8: note = Synthetic Construct
SSDFAKNF

SEQ ID NO: 87 - protein, 6 aa, synthetic construct
  REGION 1..6: note = Synthetic Construct
NQFSLK

SEQ ID NO: 88 - protein, 23 aa, synthetic construct
  REGION 1..23: note = Synthetic Construct
QGYYGMDVWGQGTTVTVSSASTK

SEQ ID NO: 89 - protein, 49 aa, synthetic construct
  REGION 1..49: note = Synthetic Construct
DYFPEPVTVSWNSGALTSGVHTFPAVLQSSGLYSLSSVVTVPSSSLGTK

SEQ ID NO: 90 - protein, 7 aa, synthetic construct
  REGION 1..7: note = Synthetic Construct
DTLMISR

SEQ ID NO: 91 - protein, 33 aa, synthetic construct
  REGION 1..33: note = Synthetic Construct
TPEVTCVVVDVSQEDPEVQFNWYVDGVEVHNAK

SEQ ID NO: 92 - protein, 16 aa, synthetic construct
  REGION 1..16: note = Synthetic Construct
VVSVLTVLHQDWLNGK

SEQ ID NO: 93 - protein, 16 aa, synthetic construct
  REGION 1..16: note = Synthetic Construct
EPQVYTLPPSQEEMTK

SEQ ID NO: 94 - protein, 10 aa, synthetic construct
  REGION 1..10: note = Synthetic Construct
NQVSLTCLVK

SEQ ID NO: 95 - protein, 22 aa, synthetic construct
  REGION 1..22: note = Synthetic Construct
GFYPSDIAVEWESNGQPENNYK

SEQ ID NO: 96 - protein, 23 aa, synthetic construct
  REGION 1..23: note = Synthetic Construct
WQEGNVFSCSVMHEALHNHYTQK

SEQ ID NO: 97 - protein, 24 aa, synthetic construct
  REGION 1..24: note = Synthetic Construct
DIVMTQSPLSLPVTPGEPASISCR

SEQ ID NO: 98 - protein, 7 aa, synthetic construct
  REGION 1..7: note = Synthetic Construct
SSQSLLR

SEQ ID NO: 99 - protein, 28 aa, synthetic construct
  REGION 1..28: note = Synthetic Construct
SNGYNYLDWYLQKPGQSPQLLIYLGSNR

SEQ ID NO: 100 - protein, 26 aa, synthetic construct
  REGION 1..26: note = Synthetic Construct
AEAEDVGVYYCMQQQEAPLTFGGGTK

SEQ ID NO: 101 - protein, 16 aa, synthetic construct
  REGION 1..16: note = Synthetic Construct
SGTASVVCLLNNFYPR

SEQ ID NO: 102 - protein, 20 aa, synthetic construct
  REGION 1..20: note = Synthetic Construct
VDNALQSGNSQESVTEQDSK

SEQ ID NO: 103 - protein, 330 aa, synthetic construct
  REGION 1..330: note = Synthetic Construct
ASTKGPSVFPLAPSSKSTSGGTAALGCLVKDYFPEPVTVSWNSGALTSGVHTFPAVLQSSGLYSLSSVVTVPSSSLGTQTYICNVNHKPSNTKVDKKVEPKSCDKTHTCPPCPAPEAAGGPSVFLFPPKPKDTLMISRTPEVTCVVVDVSHEDPEVKFNWYVDGVEVHNAKTKPREEQYNSTYRVVSVLTVLHQDWLNGKEYKCKVSNKALPASIEKTISKAKGQPREPQVYTLPPSRDELTKNQVSLTCLVKGFYPSDIAVEWESNGQPENNYKTTPPVLDSDGSFFLYSKLTVDKSRWQQGNVFSCSVMHEALHNHYTQKSLSLSPGK

SEQ ID NO: 104 - protein, 329 aa, synthetic construct
  REGION 1..329: note = Synthetic Construct
ASTKGPSVFPLAPSSKSTSGGTAALGCLVKDYFPEPVTVSWNSGALTSGVHTFPAVLQSSGLYSLSSVVTVPSSSLGTQTYICNVNHKPSNTKVDKKVEPKSCDKTHTCPPCPAPEAAGGPSVFLFPPKPKDTLMISRTPEVTCVVVDVSHEDPEVKFNWYVDGVEVHNAKTKPREEQYNSTYRVVSVLTVLHQDWLNGKEYKCKVSNKALPASIEKTISKAKGQPREPQVYTLPPSRDELTKNQVSLTCLVKGFYPSDIAVEWESNGQPENNYKTTPPVLDSDGSFFLYSKLTVDKSRWQQGNVFSCSVMHEALHNHYTQKSLSLSPG

SEQ ID NO: 105 - protein, 452 aa, synthetic construct
  REGION 1..452: note = Synthetic Construct
QVQLQESGPGLVKPSETLSLTCAVSGYSISSGYYWGWIRQPPGKGLEWIGTIYHSGSTYYNPSLKSQVTISVDTSKNQFSLELSSVTAADTAVYYCARQGSIQQGYYGMDVWGQGTTVTVSSASTKGPSVFPLAPSSKSTSGGTAALGCLVKDYFPEPVTVSWNSGALTSGVHTFPAVLQSSGLYSLSSVVTVPSSSLGTQTYICNVNHKPSNTKVDKKVEPKSCDKTHTCPPCPAPEAAGGPSVFLFPPKPKDTLMISRTPEVTCVVVDVSHEDPEVKFNWYVDGVEVHNAKTKPREEQYNSTYRVVSVLTVLHQDWLNGKEYKCKVSNKALPASIEKTISKAKGQPREPQVYTLPPSRDELTKNQVSLTCLVKGFYPSDIAVEWESNGQPENNYKTTPPVLDSDGSFFLYSKLTVDKSRWQQGNVFSCSVMHEALHNHYTQKSLSLSPGK

SEQ ID NO: 106 - protein, 451 aa, synthetic construct
  REGION 1..451: note = Synthetic Construct
QVQLQESGPGLVKPSETLSLTCAVSGYSISSGYYWGWIRQPPGKGLEWIGTIYHSGSTYYNPSLKSQVTISVDTSKNQFSLELSSVTAADTAVYYCARQGSIQQGYYGMDVWGQGTTVTVSSASTKGPSVFPLAPSSKSTSGGTAALGCLVKDYFPEPVTVSWNSGALTSGVHTFPAVLQSSGLYSLSSVVTVPSSSLGTQTYICNVNHKPSNTKVDKKVEPKSCDKTHTCPPCPAPEAAGGPSVFLFPPKPKDTLMISRTPEVTCVVVDVSHEDPEVKFNWYVDGVEVHNAKTKPREEQYNSTYRVVSVLTVLHQDWLNGKEYKCKVSNKALPASIEKTISKAKGQPREPQVYTLPPSRDELTKNQVSLTCLVKGFYPSDIAVEWESNGQPENNYKTTPPVLDSDGSFFLYSKLTVDKSRWQQGNVFSCSVMHEALHNHYTQKSLSLSPG

SEQ ID NO: 107 - protein, 122 aa, synthetic construct
  REGION 1..122: note = Synthetic Construct
QVQLQESGPGLVKPSETLSLTCAVSGYSISSVRYWGWIRQPPGKGLEWIGSIYHSGSTYYNPSLKSRVTISVDTSKNQFSLKLSSVTAADTAVYYCARQGSIKQGYYGMDVWGQGTTVTVSS

SEQ ID NO: 108 - protein, 122 aa, synthetic construct
  REGION 1..122: note = Synthetic Construct
QVQLQESGPGLVKPSETLSLTCAVSGYSISSVRYWGWIRQPPGKGLEWIGAIYPSGSTYYNPSLKSRVTISVDTSKNQFSLKLSSVTAADTAVYYCARQGSIKQGYYGMDVWGQGTTVTVSS

SEQ ID NO: 109 - protein, 122 aa, synthetic construct; identical to SEQ ID NO: 56
  REGION 1..122: note = Synthetic Construct

SEQ ID NO: 110 - protein, 122 aa, synthetic construct; identical to SEQ ID NO: 56
  REGION 1..122: note = Synthetic Construct

SEQ ID NO: 111 - protein, 122 aa, synthetic construct; identical to SEQ ID NO: 56
  REGION 1..122: note = Synthetic Construct

SEQ ID NO: 112 - protein, 122 aa, synthetic construct; identical to SEQ ID NO: 56
  REGION 1..122: note = Synthetic Construct

SEQ ID NO: 113 - protein, 112 aa, synthetic construct; identical to SEQ ID NO: 79
  REGION 1..112: note = Synthetic Construct

SEQ ID NO: 114 - protein, 112 aa, synthetic construct; identical to SEQ ID NO: 79
  REGION 1..112: note = Synthetic Construct

SEQ ID NO: 115 - protein, 112 aa, synthetic construct; identical to SEQ ID NO: 59
  REGION 1..112: note = Synthetic Construct

SEQ ID NO: 116 - protein, 112 aa, synthetic construct
  REGION 1..112: note = Synthetic Construct
DIVMTQSPLSLPVTPGESASISCRSSQGLLRSNGYNYLDWYLQKPGQSPQLLIYLGSNRASGVPDRFSGSGSGTDFTLKISRVEAEDVGVYYCMQQQETPLTFGGGTKVEIK

SEQ ID NO: 117 - protein, 112 aa, synthetic construct
  REGION 1..112: note = Synthetic Construct
DIVMTQSPLSLPVTPGEPASISCRSSQSLLRSNGYNYLDWYLQKPGQSPQLLIYLGSNRASGVPDRFSGSGSGTDFTLKISRVEAEDVGVYYCMQQQETPLTFGGGTKVEIK

SEQ ID NO: 118 - protein, 112 aa, synthetic construct
  REGION 1..112: note = Synthetic Construct
DIVMTQSPLSLPVTPGGPASISCRSSQSLLRSNGYNYLDWYLQKPGQSPQLLIYLGSNRASGVPDRFSGSGSGTDFTLKISRVEAEDVGVYYCMQQQETPLTFGGGTKVEIK

SEQ ID NO: 119 - protein, 219 aa, synthetic construct
  REGION 1..219: note = Synthetic Construct
DIVMTQSPLSLPVTPGEPASISCRSSQSLLRSHGYNYLDWYLQKPGQSPQLLIYLGSNRASGVPDRFSGSGSGTDFTLKISRAEAEDVGVYYCMQQQEAPLTFGGGTKVEIKRTVAAPSVFIFPPSDEQLKSGTASVVCLLNNFYPREAKVQWKVDNALQSGNSQESVTEQDSKDSTYSLSSTLTLSKADYEKHKVYACEVTHQGLSSPVTKSFNRGEC

SEQ ID NO: 120 - protein, 219 aa, synthetic construct
  REGION 1..219: note = Synthetic Construct
DIVMTQSPLSLPVTPGEPASISCRSSQSLLRSKGYNYLDWYLQKPGQSPQLLIYLGSNRASGVPDRFSGSGSGTDFTLKISRAEAEDVGVYYCMQQQEAPLTFGGGTKVEIKRTVAAPSVFIFPPSDEQLKSGTASVVCLLNNFYPREAKVQWKVDNALQSGNSQESVTEQDSKDSTYSLSSTLTLSKADYEKHKVYACEVTHQGLSSPVTKSFNRGEC

SEQ ID NO: 121 - protein, 219 aa, synthetic construct
  REGION 1..219: note = Synthetic Construct
DIVMTQSPLSLPVTPGEPASISCRSSQSLLRSQGYNYLDWYLQKPGQSPQLLIYLGSNRASGVPDRFSGSGSGTDFTLKISRAEAEDVGVYYCMQQQEAPLTFGGGTKVEIKRTVAAPSVFIFPPSDEQLKSGTASVVCLLNNFYPREAKVQWKVDNALQSGNSQESVTEQDSKDSTYSLSSTLTLSKADYEKHKVYACEVTHQGLSSPVTKSFNRGEC

SEQ ID NO: 122 - protein, 219 aa, synthetic construct
  REGION 1..219: note = Synthetic Construct
DIVMTQSPLSLPVTPGEPASISCRSSQSLLRSYGYNYLDWYLQKPGQSPQLLIYLGSNRASGVPDRFSGSGSGTDFTLKISRAEAEDVGVYYCMQQQEAPLTFGGGTKVEIKRTVAAPSVFIFPPSDEQLKSGTASVVCLLNNFYPREAKVQWKVDNALQSGNSQESVTEQDSKDSTYSLSSTLTLSKADYEKHKVYACEVTHQGLSSPVTKSFNRGEC

SEQ ID NO: 123 - protein, 219 aa, synthetic construct
  REGION 1..219: note = Synthetic Construct
DIVMTQSPLSLPVTPGEPASISCRSSQSLLRSEGYNYLDWYLQKPGQSPQLLIYLGSNRASGVPDRFSGSGSGTDFTLKISRAEAEDVGVYYCMQQQEAPLTFGGGTKVEIKRTVAAPSVFIFPPSDEQLKSGTASVVCLLNNFYPREAKVQWKVDNALQSGNSQESVTEQDSKDSTYSLSSTLTLSKADYEKHKVYACEVTHQGLSSPVTKSFNRGEC

SEQ ID NO: 124 - protein, 219 aa, synthetic construct
  REGION 1..219: note = Synthetic Construct
DIVMTQSPLSLPVTPGEPASISCRSSQSLLRSWGYNYLDWYLQKPGQSPQLLIYLGSNRASGVPDRFSGSGSGTDFTLKISRAEAEDVGVYYCMQQQEAPLTFGGGTKVEIKRTVAAPSVFIFPPSDEQLKSGTASVVCLLNNFYPREAKVQWKVDNALQSGNSQESVTEQDSKDSTYSLSSTLTLSKADYEKHKVYACEVTHQGLSSPVTKSFNRGEC

SEQ ID NO: 125 - protein, 219 aa, synthetic construct
  REGION 1..219: note = Synthetic Construct
DIVMTQSPLSLPVTPGEPASISCRSSQSLLRSFGYNYLDWYLQKPGQSPQLLIYLGSNRASGVPDRFSGSGSGTDFTLKISRAEAEDVGVYYCMQQQEAPLTFGGGTKVEIKRTVAAPSVFIFPPSDEQLKSGTASVVCLLNNFYPREAKVQWKVDNALQSGNSQESVTEQDSKDSTYSLSSTLTLSKADYEKHKVYACEVTHQGLSSPVTKSFNRGEC

SEQ ID NO: 126 - protein, 219 aa, synthetic construct
  REGION 1..219: note = Synthetic Construct
DIVMTQSPLSLPVTPGEPASISCRSSQSLLRSIGYNYLDWYLQKPGQSPQLLIYLGSNRASGVPDRFSGSGSGTDFTLKISRAEAEDVGVYYCMQQQEAPLTFGGGTKVEIKRTVAAPSVFIFPPSDEQLKSGTASVVCLLNNFYPREAKVQWKVDNALQSGNSQESVTEQDSKDSTYSLSSTLTLSKADYEKHKVYACEVTHQGLSSPVTKSFNRGEC

SEQ ID NO: 127 - protein, 219 aa, synthetic construct
  REGION 1..219: note = Synthetic Construct
DIVMTQSPLSLPVTPGEPASISCRSSQSLLRSVGYNYLDWYLQKPGQSPQLLIYLGSNRASGVPDRFSGSGSGTDFTLKISRAEAEDVGVYYCMQQQEAPLTFGGGTKVEIKRTVAAPSVFIFPPSDEQLKSGTASVVCLLNNFYPREAKVQWKVDNALQSGNSQESVTEQDSKDSTYSLSSTLTLSKADYEKHKVYACEVTHQGLSSPVTKSFNRGEC

SEQ ID NO: 128 - protein, 219 aa, synthetic construct
  REGION 1..219: note = Synthetic Construct
DIVMTQSPLSLPVTPGEPASISCRSSQSLLRSAGYNYLDWYLQKPGQSPQLLIYLGSNRASGVPDRFSGSGSGTDFTLKISRAEAEDVGVYYCMQQQEAPLTFGGGTKVEIKRTVAAPSVFIFPPSDEQLKSGTASVVCLLNNFYPREAKVQWKVDNALQSGNSQESVTEQDSKDSTYSLSSTLTLSKADYEKHKVYACEVTHQGLSSPVTKSFNRGEC

SEQ ID NO: 129 - protein, 219 aa, synthetic construct
  REGION 1..219: note = Synthetic Construct
DIVMTQSPLSLPVTPGEPASISCRSSQSLLRSMGYNYLDWYLQKPGQSPQLLIYLGSNRASGVPDRFSGSGSGTDFTLKISRAEAEDVGVYYCMQQQEAPLTFGGGTKVEIKRTVAAPSVFIFPPSDEQLKSGTASVVCLLNNFYPREAKVQWKVDNALQSGNSQESVTEQDSKDSTYSLSSTLTLSKADYEKHKVYACEVTHQGLSSPVTKSFNRGEC

SEQ ID NO: 130 - protein, 219 aa, synthetic construct
  REGION 1..219: note = Synthetic Construct
DIVMTQSPLSLPVTPGEPASISCRSSQSLLRSLGYNYLDWYLQKPGQSPQLLIYLGSNRASGVPDRFSGSGSGTDFTLKISRAEAEDVGVYYCMQQQEAPLTFGGGTKVEIKRTVAAPSVFIFPPSDEQLKSGTASVVCLLNNFYPREAKVQWKVDNALQSGNSQESVTEQDSKDSTYSLSSTLTLSKADYEKHKVYACEVTHQGLSSPVTKSFNRGEC

SEQ ID NO: 131 - protein, 219 aa, synthetic construct
  REGION 1..219: note = Synthetic Construct
DIVMTQSPLSLPVTPGEPASISCRSSQSLLRSNGYNYLDWYLQKPGQSPQLLIYLGSNRASGVPDRFSGSGSGTDFTLKISRVEAEDVGAYYCMQQQEAPLTFGGGTKVEIKRTVAAPSVFIFPPSDEQLKSGTASVVCLLNNFYPREAKVQWKVDNALQSGNSQESVTEQDSKDSTYSLSSTLTLSKADYEKHKVYACEVTHQGLSSPVTKSFNRGEC

SEQ ID NO: 132 - protein, 219 aa, synthetic construct
  REGION 1..219: note = Synthetic Construct
DIVMTQSPLSLPVTPGGPASISCRSSQSLLRSNGYNYLDWYLQKPGQSPQLLIYLGSNRASGVPDRLSGSGSGTDFTLKISRVEAEDVGVYYCMQQQETPLTFGGGTKVEIKRTVAAPSVFIFPPSDEQLKSGTASVVCLLNNFYPREAKVQWKVDNALQSGNSQESVTEQDSKDSTYSLSSTLTLSKADYEKHKVYACEVTHQGLSSPVTKSFNRGEC

SEQ ID NO: 133 - protein, 219 aa, synthetic construct
  REGION 1..219: note = Synthetic Construct
DIVMTQSPLSLPVTPGEPASISCRSSQSLLHSNGYNYLDWYLQKPGQSPQLLIYLGSNRASGVPDRFSGSGSGTDFTLKISRVEAEDVGVYYCMQQQETPLTFGGGTKVEIKRTVAAPSVFIFPPSDEQLKSGTASVVCLLNNFYPREAKVQWKVDNALQSGNSQESVTEQDSKDSTYSLSSTLTLSKADYEKHKVYACEVTHQGLSSPVTKSFNRGEC

SEQ ID NO: 134 - protein, 219 aa, synthetic construct
  REGION 1..219: note = Synthetic Construct
DIVMTQSPLSLPVTPGESASISCRSSQGLLRSNGYNYLDWYLQKPGQSPQLLIYLGSNRASGVPDRFSGSGSGTDFTLKISRVEAEDVGVYYCMQQQEAPLTFGGGTKVEIKRTVAAPSVFIFPPSDEQLKSGTASVVCLLNNFYPREAKVQWKVDNALQSGNSQESVTEQDSKDSTYSLSSTLTLSKADYEKHKVYACEVTHQGLSSPVTKSFNRGEC

SEQ ID NO: 135 - protein, 452 aa, synthetic construct
  REGION 1..452: note = Synthetic Construct
QVQLQESGPGLVKPSETLSLTCAVSGYSISSGYYWGWIRQPPGKGLEWIGTIYHSGSTYYNPSLESRVTISVDTSKNQFSLKLSSVTAADTAVYYCARQGSIQQGYYGMDVWGQGTTVTVSSASTKGPSVFPLAPSSKSTSGGTAALGCLVKDYFPEPVTVSWNSGALTSGVHTFPAVLQSSGLYSLSSVVTVPSSSLGTQTYICNVNHKPSNTKVDKKVEPKSCDKTHTCPPCPAPEAAGGPSVFLFPPKPKDTLMISRTPEVTCVVVDVSHEDPEVKFNWYVDGVEVHNAKTKPREEQYNSTYRVVSVLTVLHQDWLNGKEYKCKVSNKALPASIEKTISKAKGQPREPQVYTLPPSRDELTKNQVSLTCLVKGFYPSDIAVEWESNGQPENNYKTTPPVLDSDGSFFLYSKLTVDKSRWQQGNVFSCSVMHEALHNHYTQKSLSLSPGK

SEQ ID NO: 136 - protein, 451 aa, synthetic construct
  REGION 1..451: note = Synthetic Construct
QVQLQESGPGLVKPSETLSLTCAVSGYSISSGYYWGWIRQPPGKGLEWIGTIYHSGSTYYNPSLESRVTISVDTSKNQFSLKLSSVTAADTAVYYCARQGSIQQGYYGMDVWGQGTTVTVSSASTKGPSVFPLAPSSKSTSGGTAALGCLVKDYFPEPVTVSWNSGALTSGVHTFPAVLQSSGLYSLSSVVTVPSSSLGTQTYICNVNHKPSNTKVDKKVEPKSCDKTHTCPPCPAPEAAGGPSVFLFPPKPKDTLMISRTPEVTCVVVDVSHEDPEVKFNWYVDGVEVHNAKTKPREEQYNSTYRVVSVLTVLHQDWLNGKEYKCKVSNKALPASIEKTISKAKGQPREPQVYTLPPSRDELTKNQVSLTCLVKGFYPSDIAVEWESNGQPENNYKTTPPVLDSDGSFFLYSKLTVDKSRWQQGNVFSCSVMHEALHNHYTQKSLSLSPG

SEQ ID NO: 137 - protein, 452 aa, synthetic construct
  REGION 1..452: note = Synthetic Construct
QVQLQESGPGLVKPSETLSLTCAVSGYSISSGYYWGWIRQPPGKGLEWIGTIYHSGSTYYNPSLKSRVTISVDTSKNQFSLKLSSVTAADTAVYYCARQGSIKQGYYGMDVWGQGTTVTVSSASTKGPSVFPLAPSSKSTSGGTAALGCLVKDYFPEPVTVSWNSGALTSGVHTFPAVLQSSGLYSLSSVVTVPSSSLGTQTYICNVNHKPSNTKVDKKVEPKSCDKTHTCPPCPAPEAAGGPSVFLFPPKPKDTLMISRTPEVTCVVVDVSHEDPEVKFNWYVDGVEVHNAKTKPREEQYNSTYRVVSVLTVLHQDWLNGKEYKCKVSNKALPASIEKTISKAKGQPREPQVYTLPPSRDELTKNQVSLTCLVKGFYPSDIAVEWESNGQPENNYKTTPPVLDSDGSFFLYSKLTVDKSRWQQGNVFSCSVMHEALHNHYTQKSLSLSPGK

SEQ ID NO: 138 - protein, 451 aa, synthetic construct
  REGION 1..451: note = Synthetic Construct
QVQLQESGPGLVKPSETLSLTCAVSGYSISSGYYWGWIRQPPGKGLEWIGTIYHSGSTYYNPSLKSRVTISVDTSKNQFSLKLSSVTAADTAVYYCARQGSIKQGYYGMDVWGQGTTVTVSSASTKGPSVFPLAPSSKSTSGGTAALGCLVKDYFPEPVTVSWNSGALTSGVHTFPAVLQSSGLYSLSSVVTVPSSSLGTQTYICNVNHKPSNTKVDKKVEPKSCDKTHTCPPCPAPEAAGGPSVFLFPPKPKDTLMISRTPEVTCVVVDVSHEDPEVKFNWYVDGVEVHNAKTKPREEQYNSTYRVVSVLTVLHQDWLNGKEYKCKVSNKALPASIEKTISKAKGQPREPQVYTLPPSRDELTKNQVSLTCLVKGFYPSDIAVEWESNGQPENNYKTTPPVLDSDGSFFLYSKLTVDKSRWQQGNVFSCSVMHEALHNHYTQKSLSLSPG

SEQ ID NO: 139 - protein, 219 aa, synthetic construct
  REGION 1..219: note = Synthetic Construct
DIVMTQSPLSLPVTPGEPASISCRSSQSLLRSNGYNYLDWYLQKPGQSPQLLIYLGSNRASGVPDRFSGSGSGTDFTLKISRAEAEDVGVYYCMQQQEAPLTFGGGTKVEIKRTVAAPSVFIFPPSDEQLKSGTASVVCLLNNFYPREAKVQWKVDNALQSGNSQESVTEQDSKDSTYSLSSTLTLSKADYEKHKVYACEVTHQGLSSPVTKSFNRGEC

SEQ ID NO: 140 - protein, 219 aa, synthetic construct
  REGION 1..219: note = Synthetic Construct
DIVMTQSPLSLPVTPGEPASISCRSSQSLLRSNGYNYLDWYLQKPGQSPQLLIYLGSNRASGVPDRFSGSGSGTDFTLKISRVEAEDVGVYYCMQQQEAPLTFGGGTKVEIKRTVAAPSVFIFPPSDEQLKSGTASVVCLLNNFYPREAKVQWKVDNALQSGNSQESVTEQDSKDSTYSLSSTLTLSKADYEKHKVYACEVTHQGLSSPVTKSFNRGEC

SEQ ID NO: 141 - protein, 219 aa, synthetic construct
  REGION 1..219: note = Synthetic Construct
DIVMTQSPLSLPVTPGEPASISCRSSQSLLRSNGYNYLDWYLQKPGQPPQLLIYLGSNRVSGVPDRFSGSGSGTDFTLKISRVEAEDVGVYYCMQQQETPLTFGGGTKVEIKRTVAAPSVFIFPPSDEQLKSGTASVVCLLNNFYPREAKVQWKVDNALQSGNSQESVTEQDSKDSTYSLSSTLTLSKADYEKHKVYACEVTHQGLSSPVTKSFNRGEC

SEQ ID NO: 142 - protein, 219 aa, synthetic construct
  REGION 1..219: note = Synthetic Construct
DIVMTQSPLSLPVTPGEPASISCRSSQSLLRSTGYNYLDWYLQKPGQSPQLLIYLGSNRASGVPDRFSGSGSGTDFTLKISRAEAEDVGVYYCMQQQEAPLTFGGGTKVEIKRTVAAPSVFIFPPSDEQLKSGTASVVCLLNNFYPREAKVQWKVDNALQSGNSQESVTEQDSKDSTYSLSSTLTLSKADYEKHKVYACEVTHQGLSSPVTKSFNRGEC

SEQ ID NO: 143 - protein, 219 aa, synthetic construct
  REGION 1..219: note = Synthetic Construct
DIVMTQSPLSLPVTPGEPASISCRSSQSLLRSSGYNYLDWYLQKPGQSPQLLIYLGSNRASGVPDRFSGSGSGTDFTLKISRAEAEDVGVYYCMQQQEAPLTFGGGTKVEIKRTVAAPSVFIFPPSDEQLKSGTASVVCLLNNFYPREAKVQWKVDNALQSGNSQESVTEQDSKDSTYSLSSTLTLSKADYEKHKVYACEVTHQGLSSPVTKSFNRGEC

SEQ ID NO: 144 - protein, 219 aa, synthetic construct
  REGION 1..219: note = Synthetic Construct
DIVMTQSPLSLPVTPGEPASISCRSSQSLLRSGGYNYLDWYLQKPGQSPQLLIYLGSNRASGVPDRFSGSGSGTDFTLKISRAEAEDVGVYYCMQQQEAPLTFGGGTKVEIKRTVAAPSVFIFPPSDEQLKSGTASVVCLLNNFYPREAKVQWKVDNALQSGNSQESVTEQDSKDSTYSLSSTLTLSKADYEKHKVYACEVTHQGLSSPVTKSFNRGEC

SEQ ID NO: 145 - protein, 219 aa, synthetic construct
  REGION 1..219: note = Synthetic Construct
DIVMTQSPLSLPVTPGEPASISCRSSQSLLRSRGYNYLDWYLQKPGQSPQLLIYLGSNRASGVPDRFSGSGSGTDFTLKISRAEAEDVGVYYCMQQQEAPLTFGGGTKVEIKRTVAAPSVFIFPPSDEQLKSGTASVVCLLNNFYPREAKVQWKVDNALQSGNSQESVTEQDSKDSTYSLSSTLTLSKADYEKHKVYACEVTHQGLSSPVTKSFNRGEC

SEQ ID NO: 146 - protein, 219 aa, synthetic construct
  REGION 1..219: note = Synthetic Construct
DIVMTQSPLSLPVTPGEPASISCRSSQSLLRSDGYNYLDWYLQKPGQSPQLLIYLGSNRASGVPDRFSGSGSGTDFTLKISRAEAEDVGVYYCMQQQEAPLTFGGGTKVEIKRTVAAPSVFIFPPSDEQLKSGTASVVCLLNNFYPREAKVQWKVDNALQSGNSQESVTEQDSKDSTYSLSSTLTLSKADYEKHKVYACEVTHQGLSSPVTKSFNRGEC